European Patent Application EP 4 205 737 A1, published July 5, 2023. Title: Composition for preventing, improving or treating inflammatory diseases or immunological disease comprising Gancaonin N as an active ingredient. Applicant: University-Industry Cooperation Group of Kyung Hee University. The sequence listing filed with the application follows.

SEQUENCE LISTING (8 sequences)

SEQ ID NO: 1 - DNA, 22 bp, TNF-alpha Foward
gcaggtctactttgggtcattg

SEQ ID NO: 2 - DNA, 18 bp, TNF-alpha Reverse
gcgtttgggaaggttgga

SEQ ID NO: 3 - DNA, 22 bp, IL-1beta Forward
tcagccaatcttcattgctcaa

SEQ ID NO: 4 - DNA, 21 bp, IL-1beta Reverse
tggcgagctcaggtacttctg

SEQ ID NO: 5 - DNA, 20 bp, IL-6 Foward
agggctcttcggcaaatgta

SEQ ID NO: 6 - DNA, 23 bp, IL-6 Reverse
gaaggaatgcccattaacaacaa

SEQ ID NO: 7 - DNA, 19 bp, GAPDH Foward
gccacatcgctcagacacc

SEQ ID NO: 8 - DNA, 20 bp, GAPDH Reverse
cccaatacgaccaaatccgt